European Patent Application EP 4 155 405 A1, published March 29, 2023. Title: Antibody neutralizing substances substituting for function of Blood Coagulation Factor VIII. Applicant: CHUGAI SEIYAKU KABUSHIKI KAISHA. The sequence listing filed with the application follows.

SEQUENCE LISTING (182 sequences)

SEQ ID NO: 1 - protein, 118 aa, Oryctolagus cuniculus
REQLEESGGDLVKPEGSLTLTCTASGFSFSSSYWVCWVRQAPGKGLEWIGCIDTGSGNTAYASWAKGRFTISKTSSTTVTLQMTSLTAADTATYFCARGYVVAHFNLWGPGTLVTVSS

SEQ ID NO: 2 - protein, 111 aa, Oryctolagus cuniculus
ADVVMTQTPASVSEPVGGTVTIKCQASEDIERYLAWYQQKPGQPPKLLIDDASDLASGVPSRFKGSGSGTEYTLTISALECADAATYYCQSYYAISTYGVAFGGGTEVVVK

SEQ ID NO: 3 - protein, 118 aa, Oryctolagus cuniculus
QSVEESGGRLVTPGTPLTLTCTVSGFSLSSYDMSWVRQAPGKGLEYIGYITVNGVTYYANWAKGRFTISKTSTTVDLKISSPTTEDTATYFCARDQYINNGGAEFNIWGPGTLVTVSS

SEQ ID NO: 4 - protein, 110 aa, Oryctolagus cuniculus
AYDMTQTPSFVEAAVGGTVTIKCQASESISSWLSWYQQKPGQPPKLLIYQASTLASGVSSRFKGSGSGTQFTLTISDLECADAATYYCQQGYSYGDVDNAFGGGTEVVVK

SEQ ID NO: 5 - DNA, 354 bp, Oryctolagus cuniculus
cgggagcaactggaggagtccgggggagacctggtcaagcctgagggatccctgacactcacctgcacagcctctggattctccttcagtagcagctactgggtgtgctgggtccgccaggctccagggaaggggctggagtggatcggatgcattgatactggtagtggtaacactgcctacgcgagctgggcgaaaggccgattcaccatctccaagacctcgtcgaccacggtgactctgcaaatgaccagtctgacagccgcggacacggccacctatttctgtgcgagaggttatgttgttgctcactttaacttgtggggcccaggcaccctggtcaccgtctcctcc

SEQ ID NO: 6 - DNA, 333 bp, Oryctolagus cuniculus
gccgatgttgtgatgacccagactccagcctccgtgtctgaacctgtgggaggcacagtcaccatcaagtgccaggccagtgaggacattgaaaggtatttagcctggtatcagcagaaaccagggcagcctcccaagctcctgatcgatgatgcatccgatctggcatctggggtcccatcgcggttcaaaggcagtggatctgggacagaatacactctcaccatcagcgccctggagtgtgccgatgctgccacttactactgtcaaagctattatgctattagtacttatggtgttgctttcggcggagggaccgaggtggtggtcaaa

SEQ ID NO: 7 - DNA, 354 bp, Oryctolagus cuniculus
cagtcggtggaggagtccgggggtcgcctggtcacgcctgggacacccctgacactcacctgcacagtctctggattctccctcagcagctacgacatgagctgggtccgccaggctccaggaaaggggctggagtacatcggatacattactgttaatggtgtcacatactacgcgaactgggcgaaaggccgattcaccatctccaaaacctcgaccacggtggatctgaaaatctccagtccgacaaccgaggacacggccacctatttctgtgccagagatcaatatattaataatggtggtgctgaatttaacatctggggcccaggcaccctggtcaccgtctcctcc

SEQ ID NO: 8 - DNA, 330 bp, Oryctolagus cuniculus
gcctatgatatgacccagactccatccttcgtggaggcagctgtgggaggcacagtcaccatcaagtgccaggccagtgagagcattagcagttggttatcctggtatcagcagaaaccagggcagcctcccaagctcctgatctaccaggcatccactttggcatctggggtctcatcgcggttcaaaggcagtggatctgggacacagttcactctcaccatcagcgacctggagtgtgccgatgctgccacttactattgtcaacagggttatagttatggtgatgttgataatgctttcggcggagggaccgaggtggtggtcaaa

SEQ ID NO: 9 - protein, 448 aa, Artificial Sequence
  An artificially synthesized sequence
QVQLVESGGGLVQPGGSLRLSCAASGFTFSYYDIQWVRQAPGKGLEWVSSISPSGQSTYYRREVKGRFTISRDNSKNTLYLQMNSLRAEDTAVYYCARRTGREYGGGWYFDYWGQGTLVTVSSASTKGPSVFPLAPCSRSTSESTAALGCLVKDYFPEPVTVSWNSGALTSGVHTFPAVLQSSGLYSLSSVVTVPSSSLGTQTYTCNVDHKPSNTKVDKRVESKYGPPCPPCPAPEFLGGPSVFLFPPKPKDTLMISRTPEVTCVVVDVSQEDPEVQFNWYVDGVEVHNAKTKPREEQYNSTYRVVSVLTVLHQDWLNGKEYKCKVSNKGLPSSIEKTISKAKGQPREPQVYTLPPSQKEMTKNQVSLTCLVKGFYPSDIAVEWESNGQPENNYKTTPPVLDSDGSFFLYSKLTVDKSRWQEGNVFSCSVMHEALHNRYTQKSLSLSP

SEQ ID NO: 10 - protein, 214 aa, Artificial Sequence
  An artificially synthesized sequence
DIQMTQSPSSLSASVGDRVTITCKASRNIERQLAWYQQKPGQAPELLIYQASRKESGVPDRFSGSRYGTDFTLTISSLQPEDIATYYCQQYSDPPLTFGGGTKVEIKRTVAAPSVFIFPPSDEQLKSGTASVVCLLNNFYPREAKVQWKVDNALQSGNSQESVTEQDSKDSTYSLSSTLTLSKADYEKHKVYACEVTHQGLSSPVTKSFNRGEC

SEQ ID NO: 11 - protein, 444 aa, Artificial Sequence
  An artificially synthesized sequence
QVQLVQSGSELKKPGASVKVSCKASGYTFTDNNMDWVRQAPGQGLEWMGDINTRSGGSIYNEEFQDRVIMTVDKSTDTAYMELSSLRSEDTATYHCARRKSYGYYLDEWGEGTLVTVSSASTKGPSVFPLAPCSRSTSESTAALGCLVKDYFPEPVTVSWNSGALTSGVHTFPAVLQSSGLYSLSSVVTVPSSSLGTQTYTCNVDHKPSNTKVDKRVESKYGPPCPPCPAPEFLGGPSVFLFPPKPKDTLMISRTPEVTCVVVDVSQEDPEVQFNWYVDGVEVHNAKTKPREEQYNSTYRVVSVLTVLHQDWLNGKEYKCKVSNKGLPSSIEKTISKAKGQPREPQVYTLPPSQEEMTKNQVSLTCLVKGFYPSDIAVEWESNGQPENNYKTTPPVLDSDGSFFLYSKLTVDKSRWQEGNVFSCSVMHEALHNHYTQESLSLSP

SEQ ID NO: 12 - protein, 6 aa, Oryctolagus cuniculus
SSYWVC

SEQ ID NO: 13 - protein, 17 aa, Oryctolagus cuniculus
CIDTGSGNTAYASWAKG

SEQ ID NO: 14 - protein, 9 aa, Oryctolagus cuniculus
GYVVAHFNL

SEQ ID NO: 15 - DNA, 18 bp, Oryctolagus cuniculus
agcagctactgggtgtgc

SEQ ID NO: 16 - DNA, 51 bp, Oryctolagus cuniculus
tgcattgatactggtagtggtaacactgcctacgcgagctgggcgaaaggc

SEQ ID NO: 17 - DNA, 27 bp, Oryctolagus cuniculus
ggttatgttgttgctcactttaacttg

SEQ ID NO: 18 - protein, 11 aa, Oryctolagus cuniculus
QASEDIERYLA

SEQ ID NO: 19 - protein, 7 aa, Oryctolagus cuniculus
DASDLAS

SEQ ID NO: 20 - protein, 12 aa, Oryctolagus cuniculus
QSYYAISTYGVA

SEQ ID NO: 21 - DNA, 33 bp, Oryctolagus cuniculus
caggccagtgaggacattgaaaggtatttagcc

SEQ ID NO: 22 - DNA, 21 bp, Oryctolagus cuniculus
gatgcatccgatctggcatct

SEQ ID NO: 23 - DNA, 36 bp, Oryctolagus cuniculus
caaagctattatgctattagtacttatggtgttgct

SEQ ID NO: 24 - protein, 5 aa, Oryctolagus cuniculus
SYDMS

SEQ ID NO: 25 - protein, 16 aa, Oryctolagus cuniculus
YITVNGVTYYANWAKG

SEQ ID NO: 26 - protein, 13 aa, Oryctolagus cuniculus
DQYINNGGAEFNI

SEQ ID NO: 27 - DNA, 15 bp, Oryctolagus cuniculus
agctacgacatgagc

SEQ ID NO: 28 - DNA, 48 bp, Oryctolagus cuniculus
tacattactgttaatggtgtcacatactacgcgaactgggcgaaaggc

SEQ ID NO: 29 - DNA, 39 bp, Oryctolagus cuniculus
gatcaatatattaataatggtggtgctgaatttaacatc

SEQ ID NO: 30 - protein, 11 aa, Oryctolagus cuniculus
QASESISSWLS

SEQ ID NO: 31 - protein, 7 aa, Oryctolagus cuniculus
QASTLAS

SEQ ID NO: 32 - protein, 12 aa, Oryctolagus cuniculus
QQGYSYGDVDNA

SEQ ID NO: 33 - DNA, 33 bp, Oryctolagus cuniculus
caggccagtgagagcattagcagttggttatcc

SEQ ID NO: 34 - DNA, 21 bp, Oryctolagus cuniculus
caggcatccactttggcatct

SEQ ID NO: 35 - DNA, 36 bp, Oryctolagus cuniculus
caacagggttatagttatggtgatgttgataatgct

SEQ ID NO: 36 - protein, 448 aa, Artificial Sequence
  An artificially synthesized sequence
QVQLVESGGGLVQPGGSLRLSCAASGFTFSYYDINWVRQAPGKGLEWVASISPSGGSTYYRRSVKGRFTISRDNAKNSLYLQMNSLRAEDTAVYYCATRAGHNYGAGWYFDYWGQGTLVTVSSASTKGPSVFPLAPCSRSTSESTAALGCLVKDYFPEPVTVSWNSGALTSGVHTFPAVLQSSGLYSLSSVVTVPSSSLGTKTYTCNVDHKPSNTKVDKRVESKYGPPCPPCPAPEFLGGPSVFLFPPKPKDTLMISRTPEVTCVVVDVSQEDPEVQFNWYVDGVEVHNAKTKPREEQFNSTYRVVSVLTVLHQDWLNGKEYKCKVSNKGLPSSIEKTISKAKGQPREPQVCTLPPSQEEMTKNQVSLWCLVKGFYPSDIAVEWESNGQPENNYKTTPPVLDSDGSFFLYSRLTVDKSRWQEGNVFSCSVMHEALHNHYTQKSLSLSL

SEQ ID NO: 37 - protein, 444 aa, Artificial Sequence
  An artificially synthesized sequence
QVQLVQSGSELKKPGASVKVSCKASGYTFTDNNMDWVRQAPGQGLEWMGDINTRSGGSIYNEEFQDRVTMTIDKSTGTAYMELSSLRSEDTAVYYCARRRSYGYYHDEWGEGTLVTVSSASTKGPSVFPLAPCSRSTSESTAALGCLVKDYFPEPVTVSWNSGALTSGVHTFPAVLQSSGLYSLSSVVTVPSSSLGTKTYTCNVDHKPSNTKVDKRVESKYGPPCPPCPAPEFLGGPSVFLFPPKPKDTLMISRTPEVTCVVVDVSQEDPEVQFNWYVDGVEVHNAKTKPREEQFNSTYRVVSVLTVLHQDWLNGKEYKCKVSNKGLPSSIEKTISKAKGQPREPQVYTLPPSQCEMTKNQVSLSCAVKGFYPSDIAVEWESNGQPENNYKTTPPVLDSDGSFFLVSRLTVDKSRWQEGNVFSCSVMHEALHNHYTQKSLSLSL

SEQ ID NO: 38 - protein, 214 aa, Artificial Sequence
  An artificially synthesized sequence
DIQMTQSPSSLSASVGDRVTITCKASRNIERNLAWYQQKPGQAPELLIYSASRKESGVPDRFSGSRYGTDFTLTISSLQPEDLATYYCQQYYSPPLTFGGGTKVEIKRTVAAPSVFIFPPSDEQLKSGTASVVCLLNNFYPREAKVQWKVDNALQSGNSQESVTEQDSKDSTYSLSSTLTLSKADYEKHKVYACEVTHQGLSSPVTKSFNRGEC

SEQ ID NO: 39 - protein, 122 aa, Artificial Sequence
  An artificially synthesized sequence
QVQLVESGGGLVQPGGSLRLSCAASGFTFSYYDIQWVRQAPGKGLEWVSSISPSGQSTYYRREVKGRFTISRDNSKNTLYLQMNSLRAEDTAVYYCARRTGREEGGWIFDYWGQGTLVTVSS

SEQ ID NO: 40 - protein, 325 aa, Artificial Sequence
  An artificially synthesized sequence
ASTKGPSVFPLAPCSRSTSESTAALGCLVKDYFPEPVTVSWNSGALTSGVHTFPAVLKSSGLYSLSSVVTVPSSSLGTQTYTCNVDHKPSNTKVDKRVESKYGPPCPPCPAPEFLGGPSVFLFPPKPKDTLMISRTPEVTCVVVDVSQEDPEVQFNWYVDGVEVHNAKTKPREEQYNSTYRVVSVLTVLHQDWLNGKEYKCKVSNKGLPSSIEKTISKAKGQPREPQVYTLPPSQKEMTKNQVSLTCLVKGFYPSDIAVEWESNGQPENNYKTTPPVLDSDGSFFLYSRLTVDKSRWQEGNVFSCSVLHEALHAHYTRKELSLSP

SEQ ID NO: 41 - protein, 107 aa, Artificial Sequence
  An artificially synthesized sequence
EIVLTQSPATLSVSPGERATLSCRASRSVRRELAWYQQKPGQAPELLIYGASTRETGIPARFSGSGSGTDFTLTINSLEAEDAATYYCQQYRDPPGTFGGGTKVEIK

SEQ ID NO: 42 - protein, 107 aa, Artificial Sequence
  An artificially synthesized sequence
RTVAAPSVFIFPPSDEQLKSGTAEVVCLLNNFYPREAKVQWKVDNALQSGNSQESVTEQDSKDSTYSLSSTLELSKADYEKHKVYACEVTHQGLSSPVTKSFNRGEC

SEQ ID NO: 43 - protein, 119 aa, Artificial Sequence
  An artificially synthesized sequence
QVQLVQSGSELKKPGASVKVSCKASGYTFTQNNMDWVRQAPGQGLEWMGDINTRSGGVIYNEEFQDRLIMTVDKSTDTAYMELSSLRSEDTATYHCARRKSYGYYLDVWGEGTLVTVSS

SEQ ID NO: 44 - protein, 325 aa, Artificial Sequence
  An artificially synthesized sequence
ASTKGPSVFPLAPCSRSTSESTAALGCLVEDYFPEPVTVSWNSGALTSGVHTFPAVLESSGLYSLSSVVTVPSSSLGTQTYTCNVDHKPSNTKVDKRVESKYGPPCPPCPAPEFLGGPSVFLFPPKPKDTLMISRTPEVTCVVVDVSQEDPEVQFNWYVDGVEVHNAKTKPREEQYNSTYRVVSVLTVLHQDWLNGKEYKCKVSNKGLPSSIEKTISKAKGQPREPQVYTLPPSQEEMTKNQVSLTCLVKGFYPSDIAVEWESNGQPENNYKTTPPVLDSDGSFFLYSRLTVDKSRWQEGNVFSCSVLHEALHAHYTREELSLSP

SEQ ID NO: 45 - protein, 107 aa, Artificial Sequence
  An artificially synthesized sequence
SYVLTQPVSVSVALGQTATITCEGEQIGSKEVHWYHQRPGQAPILVMFRDARRPSGIPERLSGSNSGNTASLTISGAEAGDEGDYYCQVWDSSSYTVFGGGTKVTVV

SEQ ID NO: 46 - protein, 106 aa, Artificial Sequence
  An artificially synthesized sequence
GQPKAAPSVTLFPPSSEELQANKAKLVCLISDFYPGAVTVAWKADSSPVKAGVETTTPSKQSNNKYAASSYLKLTPEQWKSHRSYSCQVTHEGSTVEKTVAPTECS

SEQ ID NO: 47 - protein, 123 aa, Artificial Sequence
  An artificially synthesized sequence
QVQLVESGGGLVQPGGSLRLSCAASGFTFSYYDIQWVRQAPGKGLEWVSSISPSGQSTYYRREVKGRFTISRDNSKNTLYLQMNSLRAEDTAVYYCARRTGREYGGGWYFDYWGQGTLVTVSS

SEQ ID NO: 48 - protein, 325 aa, Artificial Sequence
  An artificially synthesized sequence
ASTKGPSVFPLAPCSRSTSESTAALGCLVKDYFPEPVTVSWNSGALTSGVHTFPAVLQSSGLYSLSSVVTVPSSSLGTQTYTCNVDHKPSNTKVDKRVESKYGPPCPPCPAPEFLGGPSVFLFPPKPKDTLMISRTPEVTCVVVDVSQEDPEVQFNWYVDGVEVHNAKTKPREEQYNSTYRVVSVLTVLHQDWLNGKEYKCKVSNKGLPSSIEKTISKAKGQPREPQVYTLPPSQKEMTKNQVSLTCLVKGFYPSDIAVEWESNGQPENNYKTTPPVLDSDGSFFLYSKLTVDKSRWQEGNVFSCSVMHEALHNRYTQKSLSLSP

SEQ ID NO: 49 - protein, 107 aa, Artificial Sequence
  An artificially synthesized sequence
DIQMTQSPSSLSASVGDRVTITCKASRNIERQLAWYQQKPGQAPELLIYQASRKESGVPDRFSGSRYGTDFTLTISSLQPEDIATYYCQQYSDPPLTFGGGTKVEIK

SEQ ID NO: 50 - protein, 107 aa, Artificial Sequence [sequence omitted]

SEQ ID NO: 51 - protein, 325 aa, Artificial Sequence
  An artificially synthesized sequence
ASTKGPSVFPLAPCSRSTSESTAALGCLVKDYFPEPVTVSWNSGALTSGVHTFPAVLQSSGLYSLSSVVTVPSSSLGTQTYTCNVDHKPSNTKVDKRVESKYGPPCPPCPAPEFRRGPSVFLFPPKPKDTLMISRTPEVTCVVVDVSQEDPEVQFNWYVDGVEVHNAKTKPREEQYNSTYRVVSVLTVLHQDWLNGKEYKCKVSNKGLPSSIEKTISKAKGQPREPQVYTLPPSQKEMTKNQVSLTCLVKGFYPSDIAVEWESNGQPENNYKTTPPVLDSDGSFFLYSRLTVDKSRWQEGNVFSCSVMHEALHNHYTQKSLSLSP

SEQ ID NO: 52 - protein, 106 aa, Artificial Sequence
  An artificially synthesized sequence
EIVLTQSPATLSVSPGERATLSCRASQSVSSNLAWYQQKPGQAPRLLIYGASTRATGIPARFSGSGSGTEFTLTISSLQSEDFAVYYCQQYKRPLTFGGGTKVEIK

SEQ ID NO: 53 - protein, 107 aa, Artificial Sequence [sequence omitted]

SEQ ID NO: 54 - protein, 106 aa, Artificial Sequence
  An artificially synthesized sequence
EIVLTQSPATLSVSPGERATLSCRASQSVRRNLAWYQQKPGQAPRLLIYGASTRATGIPARFSGSGSGTEFTLTISSLQSEDFAVYYCQQYKSPLTFGGGTKVEIK

SEQ ID NO: 55 - protein, 122 aa, Artificial Sequence
  An artificially synthesized sequence
QVQLVESGGGLVQPGGSLRLSCAASGFTFSYYDIQWVREAPGKGLEWVSSISPSGQSTYYRREVKGRFTISRDNSKNTLYLQMNSLRAEDTAVYYCARRTGREEGGWIFDYWGQGTLVTVSS

SEQ ID NO: 56 - protein, 325 aa, Artificial Sequence
  An artificially synthesized sequence
ASTKGPSVFPLAPCSRSTSESTAALGCLVKDYFPEPVTVSWNSGALTSGVHTFPAVLKSSGLYSLSSVVTVPSSSLGTQTYTCNVDHKPSNTKVDKRVESKYGPPCPPCPAPEFLGGPSVFLFPPKPKDTLMISRTPEVTCVVVDVSQEDPEVQFNWYVDGVEVHNAKTKPREEQYNSTYRVVSVLTVLHQDWLNGKEYKCKVSNKGLPSSIEKTISKAKGQPREPQVYTLPPSQKEMTKNQVSLTCLVKGFYPSDIAVEWESNGQPENNYKTTPPVLDSDGSFFLYSKLTVDKSRWQEGNVFSCSVLHEALHAHYTRKELSLSP

SEQ ID NO: 57 - protein, 107 aa, Artificial Sequence
  An artificially synthesized sequence
EIVLTQSPATLSVSPGERATLSCRASRSVRRELAWYQKKPGQAPELLIYGASTRETGIPARFSGSGSGTEFTLTISSLQSEDMAVYYCQQYRDPPGTFGGGTKVEIK

SEQ ID NO: 58 - protein, 107 aa, Artificial Sequence; identical to SEQ ID NO: 42
  An artificially synthesized sequence

SEQ ID NO: 59 - protein, 122 aa, Artificial Sequence; identical to SEQ ID NO: 39
  An artificially synthesized sequence

SEQ ID NO: 60 - protein, 107 aa, Artificial Sequence
  An artificially synthesized sequence
EIVLTQSPATLSVSPGERATLSCRASRSVRRELAWYQQKPGQAPELLIYGASTRETGIPARFSGSGSGTEFTLTISSLQSEDMAVYYCQQYRDPPGTFGGGTKVEIK

SEQ ID NO: 61 - protein, 107 aa, Artificial Sequence; identical to SEQ ID NO: 41
  An artificially synthesized sequence

SEQ ID NO: 62 - protein, 107 aa, Artificial Sequence
  An artificially synthesized sequence
EIVLTQSPATLSVSPGERATLSCRASRSVRRELAWYQKKPGQAPELLIYGASTRETGIPARFSGSGSGTDFTLTINSLEAEDAATYYCQQYRDPPGTFGGGTKVEIK

SEQ ID NO: 63 - protein, 119 aa, Artificial Sequence
  An artificially synthesized sequence
QVQLVQSGSELKKPGASVKVSCKASGYTFTDNNMDWVRQAPGQGLEWMGDINTRSGGSIYNEEFQDRVIMTVDKSTDTAYMELSSLRSEDTATYHCARRKSYGYYLDEWGEGTLVTVSS

SEQ ID NO: 64 - protein, 325 aa, Artificial Sequence
  An artificially synthesized sequence
ASTKGPSVFPLAPCSRSTSESTAALGCLVKDYFPEPVTVSWNSGALTSGVHTFPAVLQSSGLYSLSSVVTVPSSSLGTQTYTCNVDHKPSNTKVDKRVESKYGPPCPPCPAPEFLGGPSVFLFPPKPKDTLMISRTPEVTCVVVDVSQEDPEVQFNWYVDGVEVHNAKTKPREEQYNSTYRVVSVLTVLHQDWLNGKEYKCKVSNKGLPSSIEKTISKAKGQPREPQVYTLPPSQEEMTKNQVSLTCLVKGFYPSDIAVEWESNGQPENNYKTTPPVLDSDGSFFLYSKLTVDKSRWQEGNVFSCSVMHEALHNHYTQESLSLSP

SEQ ID NO: 65 - protein, 107 aa, Artificial Sequence; identical to SEQ ID NO: 49
  An artificially synthesized sequence

SEQ ID NO: 66 - protein, 107 aa, Artificial Sequence [sequence omitted]

SEQ ID NO: 67 - protein, 325 aa, Artificial Sequence
  An artificially synthesized sequence
ASTKGPSVFPLAPCSRSTSESTAALGCLVKDYFPEPVTVSWNSGALTSGVHTFPAVLQSSGLYSLSSVVTVPSSSLGTQTYTCNVDHKPSNTKVDKRVESKYGPPCPPCPAPEFRRGPSVFLFPPKPKDTLMISRTPEVTCVVVDVSQEDPEVQFNWYVDGVEVHNAKTKPREEQYNSTYRVVSVLTVLHQDWLNGKEYKCKVSNKGLPSSIEKTISKAKGQPREPQVYTLPPSQEEMTKNQVSLTCLVKGFYPSDIAVEWESNGQPENNYKTTPPVLDSDGSFFLYSRLTVDKSRWQEGNVFSCSVMHEALHNHYTQESLSLSP

SEQ ID NO: 68 - protein, 107 aa, Artificial Sequence
  An artificially synthesized sequence
SYVLTQPVSVSVARGQTATITCEGNHIGDKHVHWYHQRPGQAPILVMFRDARRPSGIPERLSGSNSGNTASLTISGAQAGDEGDYYCQVWDSSSAVVFGGGTKVTVV

SEQ ID NO: 69 - protein, 106 aa, Artificial Sequence
  An artificially synthesized sequence
GQPKAAPSVTLFPPSSEELQANKATLVCLISDFYPGAVTVAWKADSSPVKAGVETTTPSKQSNNKYAASSYLSLTPEQWKSHRSYSCQVTHEGSTVEKTVAPTECS

SEQ ID NO: 70 - protein, 107 aa, Artificial Sequence
  An artificially synthesized sequence
SYVLTQPVSVSVARGQTATITCEGNHIGDKHVHWYHQRPGQAPILVMFRDARRPSGIPERLSGSNSGNTASLTISGAQAGDEGDYYCQVWDSSSYTVFGGGTKVTVV

SEQ ID NO: 71 - protein, 119 aa, Artificial Sequence
  An artificially synthesized sequence
QVQLVQSGSELKKPGASVKVSCKASGYTFTQNNMDWVRKAPGQGLEWMGDINTRSGGVIYNEEFQDRLIMTVDKSTDTAYMELSSLRSEDTATYHCARRKSYGYYLDVWGEGTLVTVSS

SEQ ID NO: 72 - protein, 325 aa, Artificial Sequence
  An artificially synthesized sequence
ASTKGPSVFPLAPCSRSTSESTAALGCLVEDYFPEPVTVSWNSGALTSGVHTFPAVLESSGLYSLSSVVTVPSSSLGTQTYTCNVDHKPSNTKVDKRVESKYGPPCPPCPAPEFLGGPSVFLFPPKPKDTLMISRTPEVTCVVVDVSQEDPEVQFNWYVDGVEVHNAKTKPREEQYNSTYRVVSVLTVLHQDWLNGKEYKCKVSNKGLPSSIEKTISKAKGQPREPQVYTLPPSQEEMTKNQVSLTCLVKGFYPSDIAVEWESNGQPENNYKTTPPVLDSDGSFFLYSKLTVDKSRWQEGNVFSCSVLHEALHAHYTREELSLSP

SEQ ID NO: 73 - protein, 107 aa, Artificial Sequence
  An artificially synthesized sequence
SYVLTQPVSVSVALGQTATITCEGEQIGSKEVHWYHERPGQAPILVMFRDARRPSGIPERLSGSNSGNTASLTISGAEAGDEGDYYCQVWDSSSYTVFGGGTKVTVV

SEQ ID NO: 74 - protein, 106 aa, Artificial Sequence; identical to SEQ ID NO: 46
  An artificially synthesized sequence

SEQ ID NO: 75 - protein, 119 aa, Artificial Sequence; identical to SEQ ID NO: 43
  An artificially synthesized sequence

SEQ ID NO: 76 - protein, 107 aa, Artificial Sequence; identical to SEQ ID NO: 45
  An artificially synthesized sequence

SEQ ID NO: 77 - protein, 119 aa, Artificial Sequence
  An artificially synthesized sequence
QVQLVQSGSELKKPGASVKVSCKASGYTFTQNNMDWVRKAPGQGLEWMGDINTRSGGVIYNEEFQDRLIMTVDKSTDTAYMELSSLRSEDTATYHCARRKSYGYYLDEWGEGTLVTVSS

SEQ ID NO: 78 - protein, 107 aa, Artificial Sequence
  An artificially synthesized sequence
SYELTQPPSVSVALGQTATITCEGEQIGSKEVHWYHERPGQAPILVIYRDARRPSGIPERLSGSNSGNTASLTISGAEAGDEGDYYCQVWDSSSYTVFGGGTKVTVV

SEQ ID NO: 79 - protein, 124 aa, Artificial Sequence
  AQ8 VH
EVNLVESGGGLVQPGGSMSLSCAASGFTFTDYYMSWVRQPPGKALEWLALIRNKANGYTTEYSASVKGRFTISRDNSQSILYLQMNALRAEDSATYYCARDSYYSYDGYAMDYWGQGTSVTVSS

SEQ ID NO: 80 - protein, 107 aa, Artificial Sequence
  AQ8 VL
DIQMTQSPASLAASVGETITITCQASENIYFSLAWYQQKQGKSPQLLIYNTDSLKDGVPSRFSGSGSGTQYSMKINSMQPEDTATYFCRQSYDFPWTFGGGTKLEIK

SEQ ID NO: 81 - protein, 120 aa, Artificial Sequence
  AJ540 VH
QIQLVQSGPELKKPGESVKISCKASGYTFTDYAMHWVKQVPGKGLKWMGWINTYTGKPTYADDFKGRFVFSLEASASTANLQISNLKNEDTANVFCAREGGGYYWYFDFWGPGTMVTVSS

SEQ ID NO: 82 - protein, 107 aa, Artificial Sequence
  AJ540 VL
DIVMTQSPTSMSISVGDRVTMNCKANQNVDFNVDWYQQKTGQSPKLLIYKASNRYTGVPDRFTGSGSGTDFTFTISNMQAEDLAVYYCMQSNSFPLTFGSGTNLEIK

SEQ ID NO: 83 - protein, 123 aa, Artificial Sequence
  An artificially synthesized sequence
QVQLVESGGGLVQPGGSLRLSCAASGFTFSYYDIQWVRQAPGKGLEWVSSISPSGQSTYYRREVKGRFTISRDNSKNTLYLQMNSLRAEDTAVYYCARRTGREYDGGWYFDYWGQGTLVTVSS

SEQ ID NO: 84 - protein, 123 aa, Artificial Sequence
  An artificially synthesized sequence
QVQLVESGGGLVQPGGSLRLSCAASGFTFSYYDAQWVRQAPGKGLEWVSSISPSGQSTYYRREVKGRFTISRDNSKNTLYLQMNSLRAEDTAVYYCARRTGSEDGAGWYFDYWGQGTLVTVSS

SEQ ID NO: 85 - protein, 122 aa, Artificial Sequence
  An artificially synthesized sequence
QVQLVESGGGLVQPGGSLRLSCAASGFTFSYYDIQWVRQAPGKGLEWVSSISPSGQSTYYRREVKGRFTISRDNSKNTLYLQMNSLRAEDTAVYYCARRTGREDGGWHFDYWGQGTLVTVSS

SEQ ID NO: 86 - protein, 122 aa, Artificial Sequence; identical to SEQ ID NO: 55
  An artificially synthesized sequence

SEQ ID NO: 87 - protein, 122 aa, Artificial Sequence; identical to SEQ ID NO: 39
  An artificially synthesized sequence

SEQ ID NO: 88 - protein, 106 aa, Artificial Sequence
  An artificially synthesized sequence
EIVLTQSPATLSVSPGERATLSCRASQSVRRDLAWYQQKPGQAPRLLIYGASRRATGIPARFSGSGSGTEFTLTISSLQSEDFAVYYCQQYKSPLTFGGGTKVEIK

SEQ ID NO: 89 - protein, 106 aa, Artificial Sequence
  An artificially synthesized sequence
EIVLTQSPATLSVSPGERATLSCRATQSVRRDLAWYQQKPGQAPRLLIYGASRRATGIPARFSGSGSGTEFTLTISSLQSEDFAVYYCQQYRSPLTFGGGTKVEIK

SEQ ID NO: 90 - protein, 106 aa, Artificial Sequence
  An artificially synthesized sequence
EIVLTQSPATLSVSPGERATLSCRATQSVRRDLAWYQQKPGQAPELLIYGASRRATGIPARFSGSGSGTEFTLTISSLQSEDFAVYYCQQYRSPLTFGGGTKVEIK

SEQ ID NO: 91 - protein, 106 aa, Artificial Sequence
  An artificially synthesized sequence
EIVLTQSPATLSVSPGERATLSCRASRSVRRELAWYQQKPGQAPRLLIYGASTRETGIPARFSGSGSGTEFTLTISSLQSEDFAVYYCQQYRDPLTFGGGTKVEIK

SEQ ID NO: 92 - protein, 107 aa, Artificial Sequence
  An artificially synthesized sequence
EIVLTQSPATLSVSPGERATLSCRASRSVRRELAWYQKKPGQAPRLLIYGASTRETGIPDRFSGSGSGTEFTLTISSLQSEDMAVYYCQQYRDPPGTFGGGTKVEIK

SEQ ID NO: 93 - protein, 107 aa, Artificial Sequence; identical to SEQ ID NO: 57
  An artificially synthesized sequence

SEQ ID NO: 94 - protein, 107 aa, Artificial Sequence
  An artificially synthesized sequence
EIVLTQSPATLSVSPGERATLSCRATRSVRRDLAWYQKKPGQAPRLLIYGASRRETGIPDRFSGSGSGTEFTLTISSLEPEDFAVYYCQQYRDPPGTFGGGTKVEIK

SEQ ID NO: 95 - protein, 107 aa, Artificial Sequence
  An artificially synthesized sequence
EIVLTQSPATLSVSPGERATLSCRASRSVRRELAWYQKKPGQAPRLLIYGASTRETGIPDRFSGSGSGTEFTLTISSLQSEDFAVYYCQQYRDPPGTFGGGTKVEIK

SEQ ID NO: 96 - protein, 107 aa, Artificial Sequence; identical to SEQ ID NO: 60
  An artificially synthesized sequence

SEQ ID NO: 97 - protein, 107 aa, Artificial Sequence; identical to SEQ ID NO: 62
  An artificially synthesized sequence

SEQ ID NO: 98 - protein, 107 aa, Artificial Sequence; identical to SEQ ID NO: 41
  An artificially synthesized sequence

SEQ ID NO: 99 - protein, 107 aa, Artificial Sequence
  An artificially synthesized sequence
EIVLTQSPATLSVSPGERATLSCRATRSVRRDLAWYQQKPGQAPELLIYGASRRETGIPARFSGSGSGTDFTLTINSLEAEDAATYYCQQYRDPPGTFGGGTKVEIK

SEQ ID NO: 100 - protein, 119 aa, Artificial Sequence
  An artificially synthesized sequence
QVQLVQSGSELKKPGASVKVSCKASGYTFTDNNMDWVRQAPGQGLEWMGDSNTRSGTSIYNEEFQDRVIMTVDKSTDTAYMELSSLRSEDTATYHCARRKSYGYYLDEWGEGTLVTVSS

SEQ ID NO: 101 - protein, 119 aa, Artificial Sequence
  An artificially synthesized sequence
QVQLVQSGSELKKPGASVKVSCKASGYTFTNNNMDWVRQAPGQGLEWMGDINTRSGGVIYNEEFQNRVIMTVDKSTDTAYMELSSLRSEDTATYHCARRKSYGYYLDVWGEGTLVTVSS

SEQ ID NO: 102 - protein, 119 aa, Artificial Sequence
  An artificially synthesized sequence
QVQLVQSGSELKKPGASVKVSCKASGYTFTDNNMDWVRQAPGQGLEWMGDINTRSGRVISNEEFQDRVIMTVDKSTDTAYMELSSLRSEDTATYHCARRKSYGYYLDEWGEGTLVTVSS

SEQ ID NO: 103 - protein, 119 aa, Artificial Sequence
  An artificially synthesized sequence
QVQLVQSGSELKKPGASVKVSCKASGYTFTQNNMDWVRQAPGQGLEWMGDINTRSGGVIYNEEFQQRVIMTVDKSTDTAYMELSSLRSEDTATYHCARRKSYGYYLDVWGEGTLVTVSS

SEQ ID NO: 104 - protein, 119 aa, Artificial Sequence; identical to SEQ ID NO: 71
  An artificially synthesized sequence

SEQ ID NO: 105 - protein, 119 aa, Artificial Sequence
  An artificially synthesized sequence
QVQLVQSGSELKKPGASVKVSCKASGYEFTHNNMDWVRKAPGQGLEWMGDINTRSGRSIYNEEFQDRVIMTVDISTDTAYMELSSLRSEDTATYHCARRKSYGYYLDVWGEGTLVTVSS

SEQ ID NO: 106 - protein, 119 aa, Artificial Sequence; identical to SEQ ID NO: 43
  An artificially synthesized sequence

SEQ ID NO: 107 - protein, 119 aa, Artificial Sequence; identical to SEQ ID NO: 77
  An artificially synthesized sequence

SEQ ID NO: 108 - protein, 119 aa, Artificial Sequence
  An artificially synthesized sequence
QVQLVQSGSELKKPGASVKVSCKASGYTFTQNNMDWVRQAPGQGLEWMGDINTRSGGVIYNEKFQDRVIMTVDKSTDTAYMELSELRSEDTATYHCARRKSYGYYLDVWGEGTLVTVSS

SEQ ID NO: 109 - protein, 119 aa, Artificial Sequence
  An artificially synthesized sequence
QVQLVQSGSELKKPGASVKVSCKASGYEFTHNNMDWVRQAPGQGLEWMGDINTRSGRSIYNREFQDRVIMTVDISTDTAYMELSSLRSEDTATYHCARRKSYGYYLDEWGEGTLVTVSS

SEQ ID NO: 110 - protein, 119 aa, Artificial Sequence
  An artificially synthesized sequence
QVQLVQSGSELKKPGASVKVSCKASGYTFTQNNMDWVRKAPGQGLEWMGDINTRSGGVIYNEEFQDRLIMTVDKSTDTAYMELSELRSEDTATYHCARRKSYGYYLDEWGEGTLVTVSS

SEQ ID NO: 111 - protein, 107 aa, Artificial Sequence; identical to SEQ ID NO: 70
  An artificially synthesized sequence

SEQ ID NO: 112 - protein, 107 aa, Artificial Sequence
  An artificially synthesized sequence
SYVLTQPVSVSVARGQTATITCEGNHIGDKHVHWYHQRPGQAPILVMFQDARRPSGIPERLSGSNSGNTASLTISGAQAGDEGDYYCQVWDSSSYTVFGGGTKVTVV

SEQ ID NO: 113 - protein, 107 aa, Artificial Sequence
  An artificially synthesized sequence
SYVLTQPVSVSVARGQTATITCTGNHISDKHVHWYHQRPGQAPILVMFQDARRPSGIPERLSGSNSGNTASLTISGAQAGDEGDYYCQVWDSSDYTVFGGGTKVTVV

SEQ ID NO: 114 - protein, 106 aa, Artificial Sequence
  An artificially synthesized sequence
SYVLTQPVSVSVARGQTATITCEGNQISQKQVHWYHQRPGQAPILVMFRDARRPSGIPERLSGSNSGNTASLTISGAQAGDEGDYYCQVWDSSAVVFGGGTKVTVV

SEQ ID NO: 115 - protein, 107 aa, Artificial Sequence; identical to SEQ ID NO: 73
  An artificially synthesized sequence

SEQ ID NO: 116 - protein, 106 aa, Artificial Sequence
  An artificially synthesized sequence
SYVLTQPVSVSVALGQTATITCEGNQIGSREVHWYHERPGQAPILVMFRDARRPSGIPERLSGSNSGNTASLTISGAEAGDEGDYYCQVWASDAVVFGGGTKVTVV

SEQ ID NO: 117 - protein, 107 aa, Artificial Sequence; identical to SEQ ID NO: 45
  An artificially synthesized sequence

SEQ ID NO: 118 - protein, 107 aa, Artificial Sequence; identical to SEQ ID NO: 78
  An artificially synthesized sequence

SEQ ID NO: 119 - protein, 107 aa, Artificial Sequence
  An artificially synthesized sequence
SYELTQPPSVSVALGQTATITCEGEQIGSKEVHWYHQRPGQAPILVIYRDARRPSGIPERLSGSNSGNTASLTISGAEAGDEGDYYCQVWDSSSYTVFGGGTKVTVV

SEQ ID NO: 120 - protein, 106 aa, Artificial Sequence
  An artificially synthesized sequence
SYELTQPPSVSVALGQTATITCEGNQIGEKEVHWYHQRPGQAPILVMFRDARRPSGIPERLSGSNSGNTASLTISGAEAGDEGDYYCQVWASDAVVFGGGTKVTVV

SEQ ID NO: 121 - protein, 107 aa, Artificial Sequence
  An artificially synthesized sequence
SYELTQPPSVSVALGQTATITCEGEQIGSKEVHWYHERPGQAPILVMFRDARRPSGIPERLSGSNSGNTASLTISGAEAGDEGDYYCQVWDSSSYTVFGGGTKVTVV

SEQ ID NO: 122 - protein, 122 aa, Artificial Sequence
  An artificially synthesized sequence
QVQLVESGGGLVQPGGSLRLSCAASGFTFSHYDIQWVRQAPGKGLEWVSSISPSGQSTYYRREVKGRFTISRDNSKNTLYLQMNSLRAEDTAVYYCARRTDREDHGWIFDYWGQGTLVTVSS

SEQ ID NO: 123 - protein, 323 aa, Oryctolagus cuniculus
GQPKAPSVFPLAPCCGDTPSSTVTLGCLVKGYLPEPVTVTWNSGTLTNGVRTFPSVRQSSGLYSLSSVVSVTSSSQPVTCNVAHPATNTKVDKTVAPSTCSKPTCPPPELLGGPSVFIFPPKPKDTLMISRTPEVTCVVVDVSQDDPEVQFTWYINNEQVRTARPPLREQQFNSTIRVVSTLPITHQDWLRGKEFKCKVHNKALPAPIEKTISKARGQPLEPKVYTMGPPREELSSRSVSLTCMINGFYPSDISVEWEKNGKAEDNYKTTPAVLDSDGSYFLYNKLSVPTSEWQRGDVFTCSVMHEALHNHYTQKSISRSPGK

SEQ ID NO: 124 - protein, 104 aa, Oryctolagus cuniculus
GDPVAPTVLIFPPAADQVATGTVTIVCVANKYFPDVTVTWEVDGTTQTTGIENSKTPQNSADCTYNLSSTLTLTSTQYNSHKEYTCKVTQGTTSVVQSFNRGDC

SEQ ID NO: 125 - DNA, 969 bp, Oryctolagus cuniculus
gggcaacctaaggctccatcagtcttcccactggccccctgctgcggggacacacccagctccacggtgaccctgggctgcctggtcaaaggctacctcccggagccagtgaccgtgacctggaactcgggcaccctcaccaatggggtacgcaccttcccgtccgtccggcagtcctcaggcctctactcgctgagcagcgtggtgagcgtgacctcaagcagccagcccgtcacctgcaacgtggcccacccagccaccaacaccaaagtggacaagaccgttgcaccctcgacatgcagcaagcccacgtgcccaccccctgaactcctggggggaccgtctgtcttcatcttccccccaaaacccaaggacaccctcatgatctcacgcacccccgaggtcacatgcgtggtggtggacgtgagccaggatgaccccgaggtgcagttcacatggtacataaacaacgagcaggtgcgcaccgcccggccgccgctacgggagcagcagttcaacagcacgatccgcgtggtcagcaccctccccatcacgcaccaggactggctgaggggcaaggagttcaagtgcaaagtccacaacaaggcactcccggcccccatcgagaaaaccatctccaaagccagagggcagcccctggagccgaaggtctacaccatgggccctccccgggaggagctgagcagcaggtcggtcagcctgacctgcatgatcaacggcttctacccttccgacatctcggtggagtgggagaagaacgggaaggcagaggacaactacaagaccacgccggccgtgctggacagcgacggctcctacttcctctacaacaagctctcagtgcccacgagtgagtggcagcggggcgacgtcttcacctgctccgtgatgcacgaggccttgcacaaccactacacgcagaagtccatctcccgctctccgggtaaa

SEQ ID NO: 126 - DNA, 312 bp, Oryctolagus cuniculus
ggtgatccagttgcacctactgtcctcatcttcccaccagctgctgatcaggtggcaactggaacagtcaccatcgtgtgtgtggcgaataaatactttcccgatgtcaccgtcacctgggaggtggatggcaccacccaaacaactggcatcgagaacagtaaaacaccgcagaattctgcagattgtacctacaacctcagcagcactctgacactgaccagcacacagtacaacagccacaaagagtacacctgcaaggtgacccagggcacgacctcagtcgtccagagcttcaataggggtgactgt

SEQ ID NO: 127 - protein, 323 aa, Oryctolagus cuniculus; identical to SEQ ID NO: 123

SEQ ID NO: 128 - protein, 104 aa, Oryctolagus cuniculus; identical to SEQ ID NO: 124

SEQ ID NO: 129 - DNA, 969 bp, Oryctolagus cuniculus; identical to SEQ ID NO: 125

SEQ ID NO: 130 - DNA, 312 bp, Oryctolagus cuniculus; identical to SEQ ID NO: 126

SEQ ID NO: 131 - protein, 441 aa, Oryctolagus cuniculus
REQLEESGGDLVKPEGSLTLTCTASGFSFSSSYWVCWVRQAPGKGLEWIGCIDTGSGNTAYASWAKGRFTISKTSSTTVTLQMTSLTAADTATYFCARGYVVAHFNLWGPGTLVTVSSGQPKAPSVFPLAPCCGDTPSSTVTLGCLVKGYLPEPVTVTWNSGTLTNGVRTFPSVRQSSGLYSLSSVVSVTSSSQPVTCNVAHPATNTKVDKTVAPSTCSKPTCPPPELLGGPSVFIFPPKPKDTLMISRTPEVTCVVVDVSQDDPEVQFTWYINNEQVRTARPPLREQQFNSTIRVVSTLPITHQDWLRGKEFKCKVHNKALPAPIEKTISKARGQPLEPKVYTMGPPREELSSRSVSLTCMINGFYPSDISVEWEKNGKAEDNYKTTPAVLDSDGSYFLYNKLSVPTSEWQRGDVFTCSVMHEALHNHYTQKSISRSPGK

SEQ ID NO: 132 - protein, 215 aa, Oryctolagus cuniculus
ADVVMTQTPASVSEPVGGTVTIKCQASEDIERYLAWYQQKPGQPPKLLIDDASDLASGVPSRFKGSGSGTEYTLTISALECADAATYYCQSYYAISTYGVAFGGGTEVVVKGDPVAPTVLIFPPAADQVATGTVTIVCVANKYFPDVTVTWEVDGTTQTTGIENSKTPQNSADCTYNLSSTLTLTSTQYNSHKEYTCKVTQGTTSVVQSFNRGDC

SEQ ID NO: 133 - DNA, 1326 bp, Oryctolagus cuniculus
cgggagcaactggaggagtccgggggagacctggtcaagcctgagggatccctgacactcacctgcacagcctctggattctccttcagtagcagctactgggtgtgctgggtccgccaggctccagggaaggggctggagtggatcggatgcattgatactggtagtggtaacactgcctacgcgagctgggcgaaaggccgattcaccatctccaagacctcgtcgaccacggtgactctgcaaatgaccagtctgacagccgcggacacggccacctatttctgtgcgagaggttatgttgttgctcactttaacttgtggggcccaggcaccctggtcaccgtctcctccgggcaacctaaggctccatcagtcttcccactggccccctgctgcggggacacacccagctccacggtgaccctgggctgcctggtcaaaggctacctcccggagccagtgaccgtgacctggaactcgggcaccctcaccaatggggtacgcaccttcccgtccgtccggcagtcctcaggcctctactcgctgagcagcgtggtgagcgtgacctcaagcagccagcccgtcacctgcaacgtggcccacccagccaccaacaccaaagtggacaagaccgttgcaccctcgacatgcagcaagcccacgtgcccaccccctgaactcctggggggaccgtctgtcttcatcttccccccaaaacccaaggacaccctcatgatctcacgcacccccgaggtcacatgcgtggtggtggacgtgagccaggatgaccccgaggtgcagttcacatggtacataaacaacgagcaggtgcgcaccgcccggccgccgctacgggagcagcagttcaacagcacgatccgcgtggtcagcaccctccccatcacgcaccaggactggctgaggggcaaggagttcaagtgcaaagtccacaacaaggcactcccggcccccatcgagaaaaccatctccaaagccagagggcagcccctggagccgaaggtctacaccatgggccctccccgggaggagctgagcagcaggtcggtcagcctgacctgcatgatcaacggcttctacccttccgacatctcggtggagtgggagaagaacgggaaggcagaggacaactacaagaccacgccggccgtgctggacagcgacggctcctacttcctctacaacaagctctcagtgcccacgagtgagtggcagcggggcgacgtcttcacctgctccgtgatgcacgaggccttgcacaaccactacacgcagaagtccatctcccgctctccgggtaaatga

SEQ ID NO: 134 - DNA, 648 bp, Oryctolagus cuniculus
gccgatgttgtgatgacccagactccagcctccgtgtctgaacctgtgggaggcacagtcaccatcaagtgccaggccagtgaggacattgaaaggtatttagcctggtatcagcagaaaccagggcagcctcccaagctcctgatcgatgatgcatccgatctggcatctggggtcccatcgcggttcaaaggcagtggatctgggacagaatacactctcaccatcagcgccctggagtgtgccgatgctgccacttactactgtcaaagctattatgctattagtacttatggtgttgctttcggcggagggaccgaggtggtggtcaaaggtgatccagttgcacctactgtcctcatcttcccaccagctgctgatcaggtggcaactggaacagtcaccatcgtgtgtgtggcgaataaatactttcccgatgtcaccgtcacctgggaggtggatggcaccacccaaacaactggcatcgagaacagtaaaacaccgcagaattctgcagattgtacctacaacctcagcagcactctgacactgaccagcacacagtacaacagccacaaagagtacacctgcaaggtgacccagggcacgacctcagtcgtccagagcttcaataggggtgactgttag

SEQ ID NO: 135 - protein, 441 aa, Oryctolagus cuniculus
QSVEESGGRLVTPGTPLTLTCTVSGFSLSSYDMSWVRQAPGKGLEYIGYITVNGVTYYANWAKGRFTISKTSTTVDLKISSPTTEDTATYFCARDQYINNGGAEFNIWGPGTLVTVSSGQPKAPSVFPLAPCCGDTPSSTVTLGCLVKGYLPEPVTVTWNSGTLTNGVRTFPSVRQSSGLYSLSSVVSVTSSSQPVTCNVAHPATNTKVDKTVAPSTCSKPTCPPPELLGGPSVFIFPPKPKDTLMISRTPEVTCVVVDVSQDDPEVQFTWYINNEQVRTARPPLREQQFNSTIRVVSTLPITHQDWLRGKEFKCKVHNKALPAPIEKTISKARGQPLEPKVYTMGPPREELSSRSVSLTCMINGFYPSDISVEWEKNGKAEDNYKTTPAVLDSDGSYFLYNKLSVPTSEWQRGDVFTCSVMHEALHNHYTQKSISRSPGK

SEQ ID NO: 136 - protein, 214 aa, Oryctolagus cuniculus
AYDMTQTPSFVEAAVGGTVTIKCQASESISSWLSWYQQKPGQPPKLLIYQASTLASGVSSRFKGSGSGTQFTLTISDLECADAATYYCQQGYSYGDVDNAFGGGTEVVVKGDPVAPTVLIFPPAADQVATGTVTIVCVANKYFPDVTVTWEVDGTTQTTGIENSKTPQNSADCTYNLSSTLTLTSTQYNSHKEYTCKVTQGTTSVVQSFNRGDC

SEQ ID NO: 137 - DNA, 1326 bp, Oryctolagus cuniculus
cagtcggtggaggagtccgggggtcgcctggtcacgcctgggacacccctgacactcacctgcacagtctctggattctccctcagcagctacgacatgagctgggtccgccaggctccaggaaaggggctggagtacatcggatacattactgttaatggtgtcacatactacgcgaactgggcgaaaggccgattcaccatctccaaaacctcgaccacggtggatctgaaaatctccagtccgacaaccgaggacacggccacctatttctgtgccagagatcaatatattaataatggtggtgctgaatttaacatctggggcccaggcaccctggtcaccgtctcctccgggcaacctaaggctccatcagtcttcccactggccccctgctgcggggacacacccagctccacggtgaccctgggctgcctggtcaaaggctacctcccggagccagtgaccgtgacctggaactcgggcaccctcaccaatggggtacgcaccttcccgtccgtccggcagtcctcaggcctctactcgctgagcagcgtggtgagcgtgacctcaagcagccagcccgtcacctgcaacgtggcccacccagccaccaacaccaaagtggacaagaccgttgcaccctcgacatgcagcaagcccacgtgcccaccccctgaactcctggggggaccgtctgtcttcatcttccccccaaaacccaaggacaccctcatgatctcacgcacccccgaggtcacatgcgtggtggtggacgtgagccaggatgaccccgaggtgcagttcacatggtacataaacaacgagcaggtgcgcaccgcccggccgccgctacgggagcagcagttcaacagcacgatccgcgtggtcagcaccctccccatcacgcaccaggactggctgaggggcaaggagttcaagtgcaaagtccacaacaaggcactcccggcccccatcgagaaaaccatctccaaagccagagggcagcccctggagccgaaggtctacaccatgggccctccccgggaggagctgagcagcaggtcggtcagcctgacctgcatgatcaacggcttctacccttccgacatctcggtggagtgggagaagaacgggaaggcagaggacaactacaagaccacgccggccgtgctggacagcgacggctcctacttcctctacaacaagctctcagtgcccacgagtgagtggcagcggggcgacgtcttcacctgctccgtgatgcacgaggccttgcacaaccactacacgcagaagtccatctcccgctctccgggtaaatga

SEQ ID NO: 138 - DNA, 645 bp, Oryctolagus cuniculus
gcctatgatatgacccagactccatccttcgtggaggcagctgtgggaggcacagtcaccatcaagtgccaggccagtgagagcattagcagttggttatcctggtatcagcagaaaccagggcagcctcccaagctcctgatctaccaggcatccactttggcatctggggtctcatcgcggttcaaaggcagtggatctgggacacagttcactctcaccatcagcgacctggagtgtgccgatgctgccacttactattgtcaacagggttatagttatggtgatgttgataatgctttcggcggagggaccgaggtggtggtcaaaggtgatccagttgcacctactgtcctcatcttcccaccagctgctgatcaggtggcaactggaacagtcaccatcgtgtgtgtggcgaataaatactttcccgatgtcaccgtcacctgggaggtggatggcaccacccaaacaactggcatcgagaacagtaaaacaccgcagaattctgcagattgtacctacaacctcagcagcactctgacactgaccagcacacagtacaacagccacaaagagtacacctgcaaggtgacccagggcacgacctcagtcgtccagagcttcaataggggtgactgttag

SEQ ID NO: 139 - protein, 325 aa, Artificial Sequence; identical to SEQ ID NO: 56
  An artificially synthesized sequence

SEQ ID NO: 140 - protein, 107 aa, Artificial Sequence; identical to SEQ ID NO: 42
  An artificially synthesized sequence

SEQ ID NO: 141 - protein, 325 aa, Artificial Sequence; identical to SEQ ID NO: 72
  An artificially synthesized sequence

SEQ ID NO: 142 - protein, 106 aa, Artificial Sequence; identical to SEQ ID NO: 46
  An artificially synthesized sequence

SEQ ID NO: 143 - protein, 448 aa, Artificial Sequence
  An artificially synthesized sequence
QVQLVESGGGLVQPGGSLRLSCAASGFTFSYYDIQWVRQAPGKGLEWVSSISPSGQSTYYRREVKGRFTISRDNSKNTLYLQMNSLRAEDTAVYYCARRTGREYDGGWYFDYWGQGTLVTVSSASTKGPSVFPLAPCSRSTSESTAALGCLVKDYFPEPVTVSWNSGALTSGVHTFPAVLKSSGLYSLSSVVTVPSSSLGTQTYTCNVDHKPSNTKVDKRVESKYGPPCPPCPAPEFLGGPSVFLFPPKPKDTLMISRTPEVTCVVVDVSQEDPEVQFNWYVDGVEVHNAKTKPREEQYNSTYRVVSVLTVLHQDWLNGKEYKCKVSNKGLPSSIEKTISKAKGQPREPQVYTLPPSQKEMTKNQVSLTCLVKGFYPSDIAVEWESNGQPENNYKTTPPVLDSDGSFFLYSKLTVDKSRWQEGNVFSCSVLHEALHAHYTRKELSLSP

SEQ ID NO: 144 - protein, 448 aa, Artificial Sequence
  An artificially synthesized sequence
QVQLVESGGGLVQPGGSLRLSCAASGFTFSYYDAQWVRQAPGKGLEWVSSISPSGQSTYYRREVKGRFTISRDNSKNTLYLQMNSLRAEDTAVYYCARRTGSEDGAGWYFDYWGQGTLVTVSSASTKGPSVFPLAPCSRSTSESTAALGCLVKDYFPEPVTVSWNSGALTSGVHTFPAVLKSSGLYSLSSVVTVPSSSLGTQTYTCNVDHKPSNTKVDKRVESKYGPPCPPCPAPEFLGGPSVFLFPPKPKDTLMISRTPEVTCVVVDVSQEDPEVQFNWYVDGVEVHNAKTKPREEQYNSTYRVVSVLTVLHQDWLNGKEYKCKVSNKGLPSSIEKTISKAKGQPREPQVYTLPPSQKEMTKNQVSLTCLVKGFYPSDIAVEWESNGQPENNYKTTPPVLDSDGSFFLYSKLTVDKSRWQEGNVFSCSVLHEALHAHYTRKELSLSP

SEQ ID NO: 145 - protein, 447 aa, Artificial Sequence
  An artificially synthesized sequence
QVQLVESGGGLVQPGGSLRLSCAASGFTFSYYDIQWVRQAPGKGLEWVSSISPSGQSTYYRREVKGRFTISRDNSKNTLYLQMNSLRAEDTAVYYCARRTGREDGGWHFDYWGQGTLVTVSSASTKGPSVFPLAPCSRSTSESTAALGCLVKDYFPEPVTVSWNSGALTSGVHTFPAVLKSSGLYSLSSVVTVPSSSLGTQTYTCNVDHKPSNTKVDKRVESKYGPPCPPCPAPEFLGGPSVFLFPPKPKDTLMISRTPEVTCVVVDVSQEDPEVQFNWYVDGVEVHNAKTKPREEQYNSTYRVVSVLTVLHQDWLNGKEYKCKVSNKGLPSSIEKTISKAKGQPREPQVYTLPPSQKEMTKNQVSLTCLVKGFYPSDIAVEWESNGQPENNYKTTPPVLDSDGSFFLYSKLTVDKSRWQEGNVFSCSVLHEALHAHYTRKELSLSP

SEQ ID NO: 146 - protein, 447 aa, Artificial Sequence
  An artificially synthesized sequence
QVQLVESGGGLVQPGGSLRLSCAASGFTFSYYDIQWVREAPGKGLEWVSSISPSGQSTYYRREVKGRFTISRDNSKNTLYLQMNSLRAEDTAVYYCARRTGREEGGWIFDYWGQGTLVTVSSASTKGPSVFPLAPCSRSTSESTAALGCLVKDYFPEPVTVSWNSGALTSGVHTFPAVLKSSGLYSLSSVVTVPSSSLGTQTYTCNVDHKPSNTKVDKRVESKYGPPCPPCPAPEFLGGPSVFLFPPKPKDTLMISRTPEVTCVVVDVSQEDPEVQFNWYVDGVEVHNAKTKPREEQYNSTYRVVSVLTVLHQDWLNGKEYKCKVSNKGLPSSIEKTISKAKGQPREPQVYTLPPSQKEMTKNQVSLTCLVKGFYPSDIAVEWESNGQPENNYKTTPPVLDSDGSFFLYSKLTVDKSRWQEGNVFSCSVLHEALHAHYTRKELSLSP

SEQ ID NO: 147 - protein, 447 aa, Artificial Sequence
  An artificially synthesized sequence
QVQLVESGGGLVQPGGSLRLSCAASGFTFSYYDIQWVRQAPGKGLEWVSSISPSGQSTYYRREVKGRFTISRDNSKNTLYLQMNSLRAEDTAVYYCARRTGREEGGWIFDYWGQGTLVTVSSASTKGPSVFPLAPCSRSTSESTAALGCLVKDYFPEPVTVSWNSGALTSGVHTFPAVLKSSGLYSLSSVVTVPSSSLGTQTYTCNVDHKPSNTKVDKRVESKYGPPCPPCPAPEFLGGPSVFLFPPKPKDTLMISRTPEVTCVVVDVSQEDPEVQFNWYVDGVEVHNAKTKPREEQYNSTYRVVSVLTVLHQDWLNGKEYKCKVSNKGLPSSIEKTISKAKGQPREPQVYTLPPSQKEMTKNQVSLTCLVKGFYPSDIAVEWESNGQPENNYKTTPPVLDSDGSFFLYSKLTVDKSRWQEGNVFSCSVLHEALHAHYTRKELSLSP

SEQ ID NO: 148 - protein, 447 aa, Artificial Sequence
  An artificially synthesized sequence
QVQLVESGGGLVQPGGSLRLSCAASGFTFSHYDIQWVRQAPGKGLEWVSSISPSGQSTYYRREVKGRFTISRDNSKNTLYLQMNSLRAEDTAVYYCARRTDREDHGWIFDYWGQGTLVTVSSASTKGPSVFPLAPCSRSTSESTAALGCLVKDYFPEPVTVSWNSGALTSGVHTFPAVLKSSGLYSLSSVVTVPSSSLGTQTYTCNVDHKPSNTKVDKRVESKYGPPCPPCPAPEFLGGPSVFLFPPKPKDTLMISRTPEVTCVVVDVSQEDPEVQFNWYVDGVEVHNAKTKPREEQYNSTYRVVSVLTVLHQDWLNGKEYKCKVSNKGLPSSIEKTISKAKGQPREPQVYTLPPSQKEMTKNQVSLTCLVKGFYPSDIAVEWESNGQPENNYKTTPPVLDSDGSFFLYSKLTVDKSRWQEGNVFSCSVLHEALHAHYTRKELSLSP

SEQ ID NO: 149 - protein, 213 aa, Artificial Sequence
  An artificially synthesized sequence
EIVLTQSPATLSVSPGERATLSCRASQSVRRDLAWYQQKPGQAPRLLIYGASRRATGIPARFSGSGSGTEFTLTISSLQSEDFAVYYCQQYKSPLTFGGGTKVEIKRTVAAPSVFIFPPSDEQLKSGTAEVVCLLNNFYPREAKVQWKVDNALQSGNSQESVTEQDSKDSTYSLSSTLELSKADYEKHKVYACEVTHQGLSSPVTKSFNRGEC

SEQ ID NO: 150 - protein, 213 aa, Artificial Sequence
  An artificially synthesized sequence
EIVLTQSPATLSVSPGERATLSCRATQSVRRDLAWYQQKPGQAPRLLIYGASRRATGIPARFSGSGSGTEFTLTISSLQSEDFAVYYCQQYRSPLTFGGGTKVEIKRTVAAPSVFIFPPSDEQLKSGTAEVVCLLNNFYPREAKVQWKVDNALQSGNSQESVTEQDSKDSTYSLSSTLELSKADYEKHKVYACEVTHQGLSSPVTKSFNRGEC

SEQ ID NO: 151 - protein, 213 aa, Artificial Sequence
  An artificially synthesized sequence
EIVLTQSPATLSVSPGERATLSCRATQSVRRDLAWYQQKPGQAPELLIYGASRRATGIPARFSGSGSGTEFTLTISSLQSEDFAVYYCQQYRSPLTFGGGTKVEIKRTVAAPSVFIFPPSDEQLKSGTAEVVCLLNNFYPREAKVQWKVDNALQSGNSQESVTEQDSKDSTYSLSSTLELSKADYEKHKVYACEVTHQGLSSPVTKSFNRGEC

SEQ ID NO: 152 - protein, 213 aa, Artificial Sequence
  An artificially synthesized sequence
EIVLTQSPATLSVSPGERATLSCRASRSVRRELAWYQQKPGQAPRLLIYGASTRETGIPARFSGSGSGTEFTLTISSLQSEDFAVYYCQQYRDPLTFGGGTKVEIKRTVAAPSVFIFPPSDEQLKSGTAEVVCLLNNFYPREAKVQWKVDNALQSGNSQESVTEQDSKDSTYSLSSTLELSKADYEKHKVYACEVTHQGLSSPVTKSFNRGEC

SEQ ID NO: 153 - protein, 214 aa, Artificial Sequence
  An artificially synthesized sequence
EIVLTQSPATLSVSPGERATLSCRASRSVRRELAWYQKKPGQAPRLLIYGASTRETGIPDRFSGSGSGTEFTLTISSLQSEDMAVYYCQQYRDPPGTFGGGTKVEIKRTVAAPSVFIFPPSDEQLKSGTAEVVCLLNNFYPREAKVQWKVDNALQSGNSQESVTEQDSKDSTYSLSSTLELSKADYEKHKVYACEVTHQGLSSPVTKSFNRGEC

SEQ ID NO: 154 - protein, 214 aa, Artificial Sequence
  An artificially synthesized sequence
EIVLTQSPATLSVSPGERATLSCRASRSVRRELAWYQKKPGQAPELLIYGASTRETGIPARFSGSGSGTEFTLTISSLQSEDMAVYYCQQYRDPPGTFGGGTKVEIKRTVAAPSVFIFPPSDEQLKSGTAEVVCLLNNFYPREAKVQWKVDNALQSGNSQESVTEQDSKDSTYSLSSTLELSKADYEKHKVYACEVTHQGLSSPVTKSFNRGEC

SEQ ID NO: 155 - protein, 214 aa, Artificial Sequence
  An artificially synthesized sequence
EIVLTQSPATLSVSPGERATLSCRATRSVRRDLAWYQKKPGQAPRLLIYGASRRETGIPDRFSGSGSGTEFTLTISSLEPEDFAVYYCQQYRDPPGTFGGGTKVEIKRTVAAPSVFIFPPSDEQLKSGTAEVVCLLNNFYPREAKVQWKVDNALQSGNSQESVTEQDSKDSTYSLSSTLELSKADYEKHKVYACEVTHQGLSSPVTKSFNRGEC

SEQ ID NO: 156 - protein, 214 aa, Artificial Sequence
  An artificially synthesized sequence
EIVLTQSPATLSVSPGERATLSCRASRSVRRELAWYQKKPGQAPRLLIYGASTRETGIPDRFSGSGSGTEFTLTISSLQSEDFAVYYCQQYRDPPGTFGGGTKVEIKRTVAAPSVFIFPPSDEQLKSGTAEVVCLLNNFYPREAKVQWKVDNALQSGNSQESVTEQDSKDSTYSLSSTLELSKADYEKHKVYACEVTHQGLSSPVTKSFNRGEC

SEQ ID NO: 157 - protein, 214 aa, Artificial Sequence
  An artificially synthesized sequence
EIVLTQSPATLSVSPGERATLSCRASRSVRRELAWYQQKPGQAPELLIYGASTRETGIPARFSGSGSGTEFTLTISSLQSEDMAVYYCQQYRDPPGTFGGGTKVEIKRTVAAPSVFIFPPSDEQLKSGTAEVVCLLNNFYPREAKVQWKVDNALQSGNSQESVTEQDSKDSTYSLSSTLELSKADYEKHKVYACEVTHQGLSSPVTKSFNRGEC

SEQ ID NO: 158 - protein, 214 aa, Artificial Sequence
  An artificially synthesized sequence
EIVLTQSPATLSVSPGERATLSCRASRSVRRELAWYQKKPGQAPELLIYGASTRETGIPARFSGSGSGTDFTLTINSLEAEDAATYYCQQYRDPPGTFGGGTKVEIKRTVAAPSVFIFPPSDEQLKSGTAEVVCLLNNFYPREAKVQWKVDNALQSGNSQESVTEQDSKDSTYSLSSTLELSKADYEKHKVYACEVTHQGLSSPVTKSFNRGEC

SEQ ID NO: 159 - protein, 214 aa, Artificial Sequence
  An artificially synthesized sequence
EIVLTQSPATLSVSPGERATLSCRASRSVRRELAWYQQKPGQAPELLIYGASTRETGIPARFSGSGSGTDFTLTINSLEAEDAATYYCQQYRDPPGTFGGGTKVEIKRTVAAPSVFIFPPSDEQLKSGTAEVVCLLNNFYPREAKVQWKVDNALQSGNSQESVTEQDSKDSTYSLSSTLELSKADYEKHKVYACEVTHQGLSSPVTKSFNRGEC

SEQ ID NO: 160 - protein, 214 aa, Artificial Sequence
  An artificially synthesized sequence
EIVLTQSPATLSVSPGERATLSCRATRSVRRDLAWYQQKPGQAPELLIYGASRRETGIPARFSGSGSGTDFTLTINSLEAEDAATYYCQQYRDPPGTFGGGTKVEIKRTVAAPSVFIFPPSDEQLKSGTAEVVCLLNNFYPREAKVQWKVDNALQSGNSQESVTEQDSKDSTYSLSSTLELSKADYEKHKVYACEVTHQGLSSPVTKSFNRGEC

SEQ ID NO: 161 - protein, 444 aa, Artificial Sequence
  An artificially synthesized sequence
QVQLVQSGSELKKPGASVKVSCKASGYTFTDNNMDWVRQAPGQGLEWMGDSNTRSGTSIYNEEFQDRVIMTVDKSTDTAYMELSSLRSEDTATYHCARRKSYGYYLDEWGEGTLVTVSSASTKGPSVFPLAPCSRSTSESTAALGCLVEDYFPEPVTVSWNSGALTSGVHTFPAVLESSGLYSLSSVVTVPSSSLGTQTYTCNVDHKPSNTKVDKRVESKYGPPCPPCPAPEFLGGPSVFLFPPKPKDTLMISRTPEVTCVVVDVSQEDPEVQFNWYVDGVEVHNAKTKPREEQYNSTYRVVSVLTVLHQDWLNGKEYKCKVSNKGLPSSIEKTISKAKGQPREPQVYTLPPSQEEMTKNQVSLTCLVKGFYPSDIAVEWESNGQPENNYKTTPPVLDSDGSFFLYSKLTVDKSRWQEGNVFSCSVLHEALHAHYTREELSLSP

SEQ ID NO: 162 - protein, 444 aa, Artificial Sequence
  An artificially synthesized sequence
QVQLVQSGSELKKPGASVKVSCKASGYTFTNNNMDWVRQAPGQGLEWMGDINTRSGGVIYNEEFQNRVIMTVDKSTDTAYMELSSLRSEDTATYHCARRKSYGYYLDVWGEGTLVTVSSASTKGPSVFPLAPCSRSTSESTAALGCLVEDYFPEPVTVSWNSGALTSGVHTFPAVLESSGLYSLSSVVTVPSSSLGTQTYTCNVDHKPSNTKVDKRVESKYGPPCPPCPAPEFLGGPSVFLFPPKPKDTLMISRTPEVTCVVVDVSQEDPEVQFNWYVDGVEVHNAKTKPREEQYNSTYRVVSVLTVLHQDWLNGKEYKCKVSNKGLPSSIEKTISKAKGQPREPQVYTLPPSQEEMTKNQVSLTCLVKGFYPSDIAVEWESNGQPENNYKTTPPVLDSDGSFFLYSKLTVDKSRWQEGNVFSCSVLHEALHAHYTREELSLSP

SEQ ID NO: 163 - protein, 444 aa, Artificial Sequence
  An artificially synthesized sequence
QVQLVQSGSELKKPGASVKVSCKASGYTFTDNNMDWVRQAPGQGLEWMGDINTRSGRVISNEEFQDRVIMTVDKSTDTAYMELSSLRSEDTATYHCARRKSYGYYLDEWGEGTLVTVSSASTKGPSVFPLAPCSRSTSESTAALGCLVEDYFPEPVTVSWNSGALTSGVHTFPAVLESSGLYSLSSVVTVPSSSLGTQTYTCNVDHKPSNTKVDKRVESKYGPPCPPCPAPEFLGGPSVFLFPPKPKDTLMISRTPEVTCVVVDVSQEDPEVQFNWYVDGVEVHNAKTKPREEQYNSTYRVVSVLTVLHQDWLNGKEYKCKVSNKGLPSSIEKTISKAKGQPREPQVYTLPPSQEEMTKNQVSLTCLVKGFYPSDIAVEWESNGQPENNYKTTPPVLDSDGSFFLYSKLTVDKSRWQEGNVFSCSVLHEALHAHYTREELSLSP

SEQ ID NO: 164 - protein, 444 aa, Artificial Sequence
  An artificially synthesized sequence
QVQLVQSGSELKKPGASVKVSCKASGYTFTQNNMDWVRQAPGQGLEWMGDINTRSGGVIYNEEFQQRVIMTVDKSTDTAYMELSSLRSEDTATYHCARRKSYGYYLDVWGEGTLVTVSSASTKGPSVFPLAPCSRSTSESTAALGCLVEDYFPEPVTVSWNSGALTSGVHTFPAVLESSGLYSLSSVVTVPSSSLGTQTYTCNVDHKPSNTKVDKRVESKYGPPCPPCPAPEFLGGPSVFLFPPKPKDTLMISRTPEVTCVVVDVSQEDPEVQFNWYVDGVEVHNAKTKPREEQYNSTYRVVSVLTVLHQDWLNGKEYKCKVSNKGLPSSIEKTISKAKGQPREPQVYTLPPSQEEMTKNQVSLTCLVKGFYPSDIAVEWESNGQPENNYKTTPPVLDSDGSFFLYSKLTVDKSRWQEGNVFSCSVLHEALHAHYTREELSLSP

SEQ ID NO: 165 - protein, 444 aa, Artificial Sequence
  An artificially synthesized sequence
QVQLVQSGSELKKPGASVKVSCKASGYTFTQNNMDWVRKAPGQGLEWMGDINTRSGGVIYNEEFQDRLIMTVDKSTDTAYMELSSLRSEDTATYHCARRKSYGYYLDVWGEGTLVTVSSASTKGPSVFPLAPCSRSTSESTAALGCLVEDYFPEPVTVSWNSGALTSGVHTFPAVLESSGLYSLSSVVTVPSSSLGTQTYTCNVDHKPSNTKVDKRVESKYGPPCPPCPAPEFLGGPSVFLFPPKPKDTLMISRTPEVTCVVVDVSQEDPEVQFNWYVDGVEVHNAKTKPREEQYNSTYRVVSVLTVLHQDWLNGKEYKCKVSNKGLPSSIEKTISKAKGQPREPQVYTLPPSQEEMTKNQVSLTCLVKGFYPSDIAVEWESNGQPENNYKTTPPVLDSDGSFFLYSKLTVDKSRWQEGNVFSCSVLHEALHAHYTREELSLSP

SEQ ID NO: 166 - protein, 444 aa, Artificial Sequence
  An artificially synthesized sequence
QVQLVQSGSELKKPGASVKVSCKASGYEFTHNNMDWVRKAPGQGLEWMGDINTRSGRSIYNEEFQDRVIMTVDISTDTAYMELSSLRSEDTATYHCARRKSYGYYLDVWGEGTLVTVSSASTKGPSVFPLAPCSRSTSESTAALGCLVEDYFPEPVTVSWNSGALTSGVHTFPAVLESSGLYSLSSVVTVPSSSLGTQTYTCNVDHKPSNTKVDKRVESKYGPPCPPCPAPEFLGGPSVFLFPPKPKDTLMISRTPEVTCVVVDVSQEDPEVQFNWYVDGVEVHNAKTKPREEQYNSTYRVVSVLTVLHQDWLNGKEYKCKVSNKGLPSSIEKTISKAKGQPREPQVYTLPPSQEEMTKNQVSLTCLVKGFYPSDIAVEWESNGQPENNYKTTPPVLDSDGSFFLYSKLTVDKSRWQEGNVFSCSVLHEALHAHYTREELSLSP

SEQ ID NO: 167 - protein, 444 aa, Artificial Sequence
  An artificially synthesized sequence
QVQLVQSGSELKKPGASVKVSCKASGYTFTQNNMDWVRQAPGQGLEWMGDINTRSGGVIYNEEFQDRLIMTVDKSTDTAYMELSSLRSEDTATYHCARRKSYGYYLDVWGEGTLVTVSSASTKGPSVFPLAPCSRSTSESTAALGCLVEDYFPEPVTVSWNSGALTSGVHTFPAVLESSGLYSLSSVVTVPSSSLGTQTYTCNVDHKPSNTKVDKRVESKYGPPCPPCPAPEFLGGPSVFLFPPKPKDTLMISRTPEVTCVVVDVSQEDPEVQFNWYVDGVEVHNAKTKPREEQYNSTYRVVSVLTVLHQDWLNGKEYKCKVSNKGLPSSIEKTISKAKGQPREPQVYTLPPSQEEMTKNQVSLTCLVKGFYPSDIAVEWESNGQPENNYKTTPPVLDSDGSFFLYSKLTVDKSRWQEGNVFSCSVLHEALHAHYTREELSLSP

SEQ ID NO: 168 - protein, 444 aa, Artificial Sequence
  An artificially synthesized sequence
QVQLVQSGSELKKPGASVKVSCKASGYTFTQNNMDWVRKAPGQGLEWMGDINTRSGGVIYNEEFQDRLIMTVDKSTDTAYMELSSLRSEDTATYHCARRKSYGYYLDEWGEGTLVTVSSASTKGPSVFPLAPCSRSTSESTAALGCLVEDYFPEPVTVSWNSGALTSGVHTFPAVLESSGLYSLSSVVTVPSSSLGTQTYTCNVDHKPSNTKVDKRVESKYGPPCPPCPAPEFLGGPSVFLFPPKPKDTLMISRTPEVTCVVVDVSQEDPEVQFNWYVDGVEVHNAKTKPREEQYNSTYRVVSVLTVLHQDWLNGKEYKCKVSNKGLPSSIEKTISKAKGQPREPQVYTLPPSQEEMTKNQVSLTCLVKGFYPSDIAVEWESNGQPENNYKTTPPVLDSDGSFFLYSKLTVDKSRWQEGNVFSCSVLHEALHAHYTREELSLSP

SEQ ID NO: 169 - protein, 444 aa, Artificial Sequence
  An artificially synthesized sequence
QVQLVQSGSELKKPGASVKVSCKASGYTFTQNNMDWVRQAPGQGLEWMGDINTRSGGVIYNEKFQDRVIMTVDKSTDTAYMELSELRSEDTATYHCARRKSYGYYLDVWGEGTLVTVSSASTKGPSVFPLAPCSRSTSESTAALGCLVEDYFPEPVTVSWNSGALTSGVHTFPAVLESSGLYSLSSVVTVPSSSLGTQTYTCNVDHKPSNTKVDKRVESKYGPPCPPCPAPEFLGGPSVFLFPPKPKDTLMISRTPEVTCVVVDVSQEDPEVQFNWYVDGVEVHNAKTKPREEQYNSTYRVVSVLTVLHQDWLNGKEYKCKVSNKGLPSSIEKTISKAKGQPREPQVYTLPPSQEEMTKNQVSLTCLVKGFYPSDIAVEWESNGQPENNYKTTPPVLDSDGSFFLYSKLTVDKSRWQEGNVFSCSVLHEALHAHYTREELSLSP

SEQ ID NO: 170 - protein, 444 aa, Artificial Sequence
  An artificially synthesized sequence
QVQLVQSGSELKKPGASVKVSCKASGYEFTHNNMDWVRQAPGQGLEWMGDINTRSGRSIYNREFQDRVIMTVDISTDTAYMELSSLRSEDTATYHCARRKSYGYYLDEWGEGTLVTVSSASTKGPSVFPLAPCSRSTSESTAALGCLVEDYFPEPVTVSWNSGALTSGVHTFPAVLESSGLYSLSSVVTVPSSSLGTQTYTCNVDHKPSNTKVDKRVESKYGPPCPPCPAPEFLGGPSVFLFPPKPKDTLMISRTPEVTCVVVDVSQEDPEVQFNWYVDGVEVHNAKTKPREEQYNSTYRVVSVLTVLHQDWLNGKEYKCKVSNKGLPSSIEKTISKAKGQPREPQVYTLPPSQEEMTKNQVSLTCLVKGFYPSDIAVEWESNGQPENNYKTTPPVLDSDGSFFLYSKLTVDKSRWQEGNVFSCSVLHEALHAHYTREELSLSP

SEQ ID NO: 171 - protein, 444 aa, Artificial Sequence
  An artificially synthesized sequence
QVQLVQSGSELKKPGASVKVSCKASGYTFTQNNMDWVRKAPGQGLEWMGDINTRSGGVIYNEEFQDRLIMTVDKSTDTAYMELSELRSEDTATYHCARRKSYGYYLDEWGEGTLVTVSSASTKGPSVFPLAPCSRSTSESTAALGCLVEDYFPEPVTVSWNSGALTSGVHTFPAVLESSGLYSLSSVVTVPSSSLGTQTYTCNVDHKPSNTKVDKRVESKYGPPCPPCPAPEFLGGPSVFLFPPKPKDTLMISRTPEVTCVVVDVSQEDPEVQFNWYVDGVEVHNAKTKPREEQYNSTYRVVSVLTVLHQDWLNGKEYKCKVSNKGLPSSIEKTISKAKGQPREPQVYTLPPSQEEMTKNQVSLTCLVKGFYPSDIAVEWESNGQPENNYKTTPPVLDSDGSFFLYSKLTVDKSRWQEGNVFSCSVLHEALHAHYTREELSLSP

SEQ ID NO: 172 - protein, 213 aa, Artificial Sequence
  An artificially synthesized sequence
SYVLTQPVSVSVARGQTATITCEGNHIGDKHVHWYHQRPGQAPILVMFRDARRPSGIPERLSGSNSGNTASLTISGAQAGDEGDYYCQVWDSSSYTVFGGGTKVTVVGQPKAAPSVTLFPPSSEELQANKAKLVCLISDFYPGAVTVAWKADSSPVKAGVETTTPSKQSNNKYAASSYLKLTPEQWKSHRSYSCQVTHEGSTVEKTVAPTECS

SEQ ID NO: 173 - protein, 213 aa, Artificial Sequence
  An artificially synthesized sequence
SYVLTQPVSVSVARGQTATITCEGNHIGDKHVHWYHQRPGQAPILVMFQDARRPSGIPERLSGSNSGNTASLTISGAQAGDEGDYYCQVWDSSSYTVFGGGTKVTVVGQPKAAPSVTLFPPSSEELQANKAKLVCLISDFYPGAVTVAWKADSSPVKAGVETTTPSKQSNNKYAASSYLKLTPEQWKSHRSYSCQVTHEGSTVEKTVAPTECS

SEQ ID NO: 174 - protein, 213 aa, Artificial Sequence
  An artificially synthesized sequence
SYVLTQPVSVSVARGQTATITCTGNHISDKHVHWYHQRPGQAPILVMFQDARRPSGIPERLSGSNSGNTASLTISGAQAGDEGDYYCQVWDSSDYTVFGGGTKVTVVGQPKAAPSVTLFPPSSEELQANKAKLVCLISDFYPGAVTVAWKADSSPVKAGVETTTPSKQSNNKYAASSYLKLTPEQWKSHRSYSCQVTHEGSTVEKTVAPTECS

SEQ ID NO: 175 - protein, 212 aa, Artificial Sequence
  An artificially synthesized sequence
SYVLTQPVSVSVARGQTATITCEGNQISQKQVHWYHQRPGQAPILVMFRDARRPSGIPERLSGSNSGNTASLTISGAQAGDEGDYYCQVWDSSAVVFGGGTKVTVVGQPKAAPSVTLFPPSSEELQANKAKLVCLISDFYPGAVTVAWKADSSPVKAGVETTTPSKQSNNKYAASSYLKLTPEQWKSHRSYSCQVTHEGSTVEKTVAPTECS

SEQ ID NO: 176 - protein, 213 aa, Artificial Sequence
  An artificially synthesized sequence
SYVLTQPVSVSVALGQTATITCEGEQIGSKEVHWYHERPGQAPILVMFRDARRPSGIPERLSGSNSGNTASLTISGAEAGDEGDYYCQVWDSSSYTVFGGGTKVTVVGQPKAAPSVTLFPPSSEELQANKAKLVCLISDFYPGAVTVAWKADSSPVKAGVETTTPSKQSNNKYAASSYLKLTPEQWKSHRSYSCQVTHEGSTVEKTVAPTECS

SEQ ID NO: 177 - protein, 212 aa, Artificial Sequence
  An artificially synthesized sequence
SYVLTQPVSVSVALGQTATITCEGNQIGSREVHWYHERPGQAPILVMFRDARRPSGIPERLSGSNSGNTASLTISGAEAGDEGDYYCQVWASDAVVFGGGTKVTVVGQPKAAPSVTLFPPSSEELQANKAKLVCLISDFYPGAVTVAWKADSSPVKAGVETTTPSKQSNNKYAASSYLKLTPEQWKSHRSYSCQVTHEGSTVEKTVAPTECS

SEQ ID NO: 178 - protein, 213 aa, Artificial Sequence
  An artificially synthesized sequence
SYVLTQPVSVSVALGQTATITCEGEQIGSKEVHWYHQRPGQAPILVMFRDARRPSGIPERLSGSNSGNTASLTISGAEAGDEGDYYCQVWDSSSYTVFGGGTKVTVVGQPKAAPSVTLFPPSSEELQANKAKLVCLISDFYPGAVTVAWKADSSPVKAGVETTTPSKQSNNKYAASSYLKLTPEQWKSHRSYSCQVTHEGSTVEKTVAPTECS

SEQ ID NO: 179 - protein, 213 aa, Artificial Sequence
  An artificially synthesized sequence
SYELTQPPSVSVALGQTATITCEGEQIGSKEVHWYHERPGQAPILVIYRDARRPSGIPERLSGSNSGNTASLTISGAEAGDEGDYYCQVWDSSSYTVFGGGTKVTVVGQPKAAPSVTLFPPSSEELQANKAKLVCLISDFYPGAVTVAWKADSSPVKAGVETTTPSKQSNNKYAASSYLKLTPEQWKSHRSYSCQVTHEGSTVEKTVAPTECS

SEQ ID NO: 180 - protein, 213 aa, Artificial Sequence
  An artificially synthesized sequence
SYELTQPPSVSVALGQTATITCEGEQIGSKEVHWYHQRPGQAPILVIYRDARRPSGIPERLSGSNSGNTASLTISGAEAGDEGDYYCQVWDSSSYTVFGGGTKVTVVGQPKAAPSVTLFPPSSEELQANKAKLVCLISDFYPGAVTVAWKADSSPVKAGVETTTPSKQSNNKYAASSYLKLTPEQWKSHRSYSCQVTHEGSTVEKTVAPTECS

SEQ ID NO: 181 - protein, 212 aa, Artificial Sequence
  An artificially synthesized sequence
SYELTQPPSVSVALGQTATITCEGNQIGEKEVHWYHQRPGQAPILVMFRDARRPSGIPERLSGSNSGNTASLTISGAEAGDEGDYYCQVWASDAVVFGGGTKVTVVGQPKAAPSVTLFPPSSEELQANKAKLVCLISDFYPGAVTVAWKADSSPVKAGVETTTPSKQSNNKYAASSYLKLTPEQWKSHRSYSCQVTHEGSTVEKTVAPTECS

SEQ ID NO: 182 - protein, 213 aa, Artificial Sequence
  An artificially synthesized sequence
SYELTQPPSVSVALGQTATITCEGEQIGSKEVHWYHERPGQAPILVMFRDARRPSGIPERLSGSNSGNTASLTISGAEAGDEGDYYCQVWDSSSYTVFGGGTKVTVVGQPKAAPSVTLFPPSSEELQANKAKLVCLISDFYPGAVTVAWKADSSPVKAGVETTTPSKQSNNKYAASSYLKLTPEQWKSHRSYSCQVTHEGSTVEKTVAPTECS